European Patent Specification EP 3 740 225 B1, published September 10, 2025. Title: Viral treatment. Applicant: Pneumagen Ltd Connaris, Helen Yang, Lei Potter, Jane. The sequence listing filed with the application follows.

SEQUENCE LISTING (31 sequences)

SEQ ID NO: 1 - protein, 781 aa, Vibrio cholerae
MRFKNVKKTALMLAMFGMATSSNAALFDYNATGDTEFDSPAKQGWMQDNTNNGSGVLTNADGMPAWLVQGIGGRAQWTYSLSTNQHAQASSFGWRMTTEMKVLSGGMITNYYANGTQRVLPIISLDSSGNLVVEFEGQTGRTVLATGTAATEYHKFELVFLPGSNPSASFYFDGKLIRDNIQPTASKQNMIVWGNGSSNTDGVAAYRDIKFEIQGDVIFRGPDRIPSIVASSVTPGVVTAFAEKRVGGGDPGALSNTNDIITRTSRDGGITWDTELNLTEQINVSDEFDFSDPRPIYDPSSNTVLVSYARWPTDAAQNGDRIKPWMPNGIFYSVYDVASGNWQAPIDVTDQVKERSFQIAGWGGSELYRRNTSLNSQQDWQSNAKIRIVDGAANQIQVADGSRKYVVTLSIDESGGLVANLNGVSAPIILQSEHAKVHSFHDYELQYSALNHTTTLFVDGQQITTWAGEVSQENNIQFGNADAQIDGRLHVQKIVLTQQGHNLVEFDAFYLAQQTPEVEKDLEKLGWTKIKTGNTMSLYGNASVNPGPGHGITLTRQQNISGSQNGRLIYPAIVLDRFFLNVMSIYSDDGGSNWQTGSTLPIPFRWKSSSILETLEPSEADMVELQNGDLLLTARLDFNQIVNGVNYSPRQQFLSKDGGITWSLLEANNANVFSNISTGTVDASITRFEQSDGSHFLLFTNPQGNPAGTNGRQNLGLWFSFDEGVTWKGPIQLVNGASAYSDIYQLDSENAIVIVETDNSNMRILRMPITLLKQKLTLSQN

SEQ ID NO: 2 - protein, 176 aa, Vibrio cholerae
ALFDYNATGDTEFDSPAKQGWMQDNTNNGSGVLTNADGMPAWLVQGIGGRAQWTYSLSTNQHAQASSFGWRMTTEMKVLSGGMITNYYANGTQRVLPIISLDSSGNLVVEFEGQTGRTVLATGTAATEYHKFELVFLPGSNPSASFYFDGKLIRDNIQPTASKQNMIVWGNGSSNT

SEQ ID NO: 3 - protein, 1035 aa, Streptococcus pneumoniae
MSYFRNRDIDIERNSMNRSVQERKCRYSIRKLSVGAVSMIVGAVVFGTSPVLAQEGASEQPLANETQLSGESSTLTDTEKSQPSSETELSGNKQEQERKDKQEEKIPRDYYARDLENVETVIEKEDVETNASNGQRVDLSSELDKLKKLENATVHMEFKPDAKAPAFYNLFSVSSATKKDEYFTMAVYNNTATLEGRGSDGKQFYNNYNDAPLKVKPGQWNSVTFTVEKPTAELPKGRVRLYVNGVLSRTSLRSGNFIKDMPDVTHVQIGATKRANNTVWGSNLQIRNLTVYNRALTPEEVQKRSQLFKRSDLEKKLPEGAALTEKTDIFESGRNGKPNKDGIKSYRIPALLKTDKGTLIAGADERRLHSSDWGDIGMVIRRSEDNGKTWGDRVTITNLRDNPKASDPSIGSPVNIDMVLVQDPETKRIFSIYDMFPEGKGIFGMSSQKEEAYKKIDGKTYQILYREGEKGAYTIRENGTVYTPDGKATDYRVVVDPVKPAYSDKGDLYKGNQLLGNIYFTTNKTSPFRIAKDSYLWMSYSDDDGKTWSAPQDITPMVKADWMKFLGVGPGTGIVLRNGPHKGRILIPVYTTNNVSHLNGSQSSRIIYSDDHGKTWHAGEAVNDNRQVDGQKIHSSTMNNRRAQNTESTVVQLNNGDVKLFMRGLTGDLQVATSKDGGVTWEKDIKRYPQVKDVYVQMSAIHTMHEGKEYIILSNAGGPKRENGMVHLARVEENGELTWLKHNPIQKGEFAYNSLQELGNGEYGILYEHTEKGQNAYTLSFRKFNWDFLSKDLISPTEAKVKRTREMGKGVIGLEFDSEVLVNKAPTLQLANGKTARFMTQYDTKTLLFTVDSEDMGQKVTGLAEGAIESMHNLPVSVAGTKLSNGMNGSEAAVHEVPEYTGPLGTSGEEPAPTVEKPEYTGPLGTSGEEPAPTVEKPEYTGPLGTAGEEAAPTVEKPEFTGGVNGTEPAVHEIAEYKGSDSLVTLTTKEDYTYKAPLAQQALPETGNKESDLLASLGLTAFFLGLFTLGKKREQ

SEQ ID NO: 4 - protein, 185 aa, Streptococcus pneumoniae
FMRGLTGDLQVATSKDGGVTWEKDIKRYPQVKDVYVQMSAIHTMHEGKEYIILSNAGGPKRENGMVHLARVEENGELTWLKHNPIQKGEFAYNSLQELGNGEYGILYEHTEKGQNAYTLSFRKFNWDFLSKDLISPTEAKVKRTREMGKGVIGLEFDSEVLVNKAPTLQLANGKTARFMTQYDTK

SEQ ID NO: 5 - protein, 438 aa, Pseudomonas aeruginosa
MNTYFDIPHRLVGKALYESYYDHFGQMDILSDGSLYLIYRRATEHVGGSDGRVVFSKLEGGIWSAPTIVAQAGGQDFRDVAGGTMPSGRIVAASTVYETGEVKVYVSDDSGVTWVHKFTLARGGADYNFAHGKSFQVGARYVIPLYAATGVNYELKWLESSDGGETWGEGSTIYSGNTPYNETSYLPVGDGVILAVARVGSGAGGALRQFISLDDGGTWTDQGNVTAQNGDSTDILVAPSLSYIYSEGGTPHVVLLYTNRTTHFCYYRTILLAKAVAGSSGWTERVPVYSAPAASGYTSQVVLGGRRILGNLFRETSSTTSGAYQFEVYLGGVPDFESDWFSVSSNSLYTLSHGLQRSPRRVVVEFARSSSPSTWNIVMPSYFNDGGHKGSGAQVEVGSLNIRLGTGAAVWGTGYFGGIDNSATTRFATGYYRVRAWI

SEQ ID NO: 6 - protein, 106 aa, Pseudomonas aeruginosa
VPDFESDWFSVSSNSLYTLSHGLQRSPRRVVVEFARSSSPSTWNIVMPSYFNDGGHKGSGAQVEVGSLNIRLGTGAAVWGTGYFGGIDNSATTRFATGYYRVRAWI

SEQ ID NO: 7 - protein, 489 aa, Streptococcus pneumoniae
GAMVIEKEDVETNASNGQRVDLSSELDKLKKLENATVHMEFKPDAKAPAFYNLFSVSSATKKDEYFTMAVYNNTATLEGRGSDGKQFYNNYNDAPLKVKPGQWNSVTFTVEKPTAELPKGRVRLYVNGVLSRTSLRSGNFIKDMPDVTHVQIGATKRANNTVWGSNLQIRNLTVYNRALTPEEVQKRSGGGSGVIEKEDVETNASNGQRVDLSSELDKLKKLENATVHMEFKPDAKAPAFYNLFSVSSATKKDEYFTMAVYNNTATLEGRGSDGKQFYNNYNDAPLKVKPGQWNSVTFTVEKPTAELPKGRVRLYVNGVLSRTSLRSGNFIKDMPDVTHVQIGATKRANNTVWGSNLQIRNLTVYNRALTPEEVQKRSGGALGVPDFESDWFSVSSNSLYTLSHGLQRSPRRVVVEFARSSSPSTWNIVMPSYFNDGGHKGSGAQVEVGSLNIRLGTGAAVWGTGYFGGIDNSATTRFATGYYRVRAWI

SEQ ID NO: 8 - protein, 489 aa, Artificial Sequence
  Modified CBM
GAMVIEKEDVETNASNGQRVDLSSELDKLKKLENATVHMEFKPDAKAPAFYNLFSVSSATKKDEYFTMAVYNNTATLEGRGSDGKQFYNNYNDAPLKVKPGQWNSVTFTVEKPTAELPKGRARLYVNGGLSRTSLRSGNFIKDMPDVTHVQIGATKRANNTVWGSNLQIRNLTVYNRALTPEEVQKRSGGGSGVIEKEDVETNASNGQRVDLSSELDKLKKLENATVHMEFKPDAKAPAFYNLFSVSSATKKDEYFTMAVYNNTATLEGRGSDGKQFYNNYNDAPLKVKPGQWNSVTFTVEKPTAELPKGRARLYVNGGLSRTSLRSGNFIKDMPDVTHVQIGATKRANNTVWGSNLQIRNLTVYNRALTPEEVQKRSGGSLGVPDFESDWFDVSSNSLYTLSHGLQRSPRRVVVEFARSSSPSTWNIVMPSYFNDGGHKGSGAQVEVGSLNIKLGTGAAVWGTGYFGGIDNSATTRFATGYYRVRAWI

SEQ ID NO: 9 - protein, 489 aa, Artificial Sequence
  Modified CBM
GAMVIEKEDVETNASNGQRVDLSSELDKLKKLENATVHMEFKPDPKAPAFYNLFSVSSATKKDEYFTMAVYNNTATLEGRGSDGKQFYNNYNDAPLKVKPGQWNSVTFTVEKPTAELPKGRARLYVNGGLSRTSLRSGNFIKDMPDVTHVQIGATKRANNTVWGSNLQIRNLTVYNRALTPEEVQKRSGGGSGVIEKEDVETNASNGQRVDLSSELDKLKKLENATVHMEFKPDPKAPAFYNLFSVSSATKKDEYFTMAVYNNTATLEGRGSDGKQFYNNYNDAPLKVKPGQWNSVTFTVEKPTAELPKGRARLYVNGGLSRTSLRSGNFIKDMPDVTHVQIGATKRANNTVWGSNLQIRNLTVYNRALTPEEVQKRSGGSLGVPDFESDWFDVSSNSLYTLSHGLQRSPRRVVVEFARSSSPSTWNIVMPSYFNDGGHKGSGAQVEVGSLNIKLGTGAAVWGTGYFGGIDNSATTRFATGYYRVRAWI

SEQ ID NO: 10 - protein, 393 aa, Artificial Sequence
  Vc2CBM
GAMALFDYNATGDTEFDSPAKQGWMQDNTNNGSGVLTNADGMPAWLVQGIGGRAQWTYSLSTNQHAQASSFGWRMTTEMKVLSGGMITNYYANGTQRVLPIISLDSSGNLVVEFEGQTGRTVLATGTAATEYHKFELVFLPGSNPSASFYFDGKLIRDNIQPTASKQNMIVWGNGSSNTDGVAAYRDIKFEIQGDALNGSMALFDYNATGDTEFDSPAKQGWMQDNTNNGSGVLTNADGMPAWLVQGIGGRAQWTYSLSTNQHAQASSFGWRMTTEMKVLSGGMITNYYANGTQRVLPIISLDSSGNLVVEFEGQTGRTVLATGTAATEYHKFELVFLPGSNPSASFYFDGKLIRDNIQPTASKQNMIVWGNGSSNTDGVAAYRDIKFEIQGD

SEQ ID NO: 11 - protein, 789 aa, Artificial Sequence
  Vc4CBM
GAMALFDYNATGDTEFDSPAKQGWMQDNTNNGSGVLTNADGMPAWLVQGIGGRAQWTYSLSTNQHAQASSFGWRMTTEMKVLSGGMITNYYANGTQRVLPIISLDSSGNLVVEFEGQTGRTVLATGTAATEYHKFELVFLPGSNPSASFYFDGKLIRDNIQPTASKQNMIVWGNGSSNTDGVAAYRDIKFEIQGDALNGSMALFDYNATGDTEFDSPAKQGWMQDNTNNGSGVLTNADGMPAWLVQGIGGRAQWTYSLSTNQHAQASSFGWRMTTEMKVLSGGMITNYYANGTQRVLPIISLDSSGNLVVEFEGQTGRTVLATGTAATEYHKFELVFLPGSNPSASFYFDGKLIRDNIQPTASKQNMIVWGNGSSNTDGVAAYRDIKFEIQGDLQALGMALFDYNATGDTEFDSPAKQGWMQDNTNNGSGVLTNADGMPAWLVQGIGGRAQWTYSLSTNQHAQASSFGWRMTTEMKVLSGGMITNYYANGTQRVLPIISLDSSGNLVVEFEGQTGRTVLATGTAATEYHKFELVFLPGSNPSASFYFDGKLIRDNIQPTASKQNMIVWGNGSSNTDGVAAYRDIKFEIQGDGGNSGMALFDYNATGDTEFDSPAKQGWMQDNTNNGSGVLTNADGMPAWLVQGIGGRAQWTYSLSTNQHAQASSFGWRMTTEMKVLSGGMITNYYANGTQRVLPIISLDSSGNLVVEFEGQTGRTVLATGTAATEYHKFELVFLPGSNPSASFYFDGKLIRDNIQPTASKQNMIVWGNGSSNTDGVAAYRDIKFEIQGD

SEQ ID NO: 12 - protein, 188 aa, Streptococcus pneumoniae
GSMVIEKEDVETNASNGQRVDLSSELDKLKKLENATVHMEFKPDAKAPAFYNLFSVSSATKKDEYFTMAVYNNTATLEGRGSDGKQFYNNYNDAPLKVKPGQWNSVTFTVEKPTAELPKGRVRLYVNGVLSRTSLRSGNFIKDMPDVTHVQIGATKRANNTVWGSNLQIRNLTVYNRALTPEEVQKRS

SEQ ID NO: 13 - protein, 5 aa, Artificial Sequence
  Peptide linker
  MISC_FEATURE (3)..(3): x = any amino acid
ALXGS

SEQ ID NO: 14 - protein, 5 aa, Artificial Sequence
  Peptide linker
LQALG

SEQ ID NO: 15 - protein, 5 aa, Artificial Sequence
  Peptide linker
  MISC_FEATURE (3)..(3): x = any amino acid
GGXSG

SEQ ID NO: 16 - protein, 5 aa, Artificial Sequence
  Peptide linker
GGALG

SEQ ID NO: 17 - protein, 5 aa, Artificial Sequence
  Peptide linker
GGGGS

SEQ ID NO: 18 - protein, 10 aa, Artificial Sequence
  Peptide linker
  MISC_FEATURE (3)..(3): x = any amino acid
ALXGSGGGSG

SEQ ID NO: 19 - protein, 10 aa, Artificial Sequence
  Peptide linker
LQALGGGGSL

SEQ ID NO: 20 - protein, 15 aa, Artificial Sequence
  Peptide linker
  MISC_FEATURE (3)..(3): X = any amino acid
ALXGSGGGSGGGGSG

SEQ ID NO: 21 - protein, 10 aa, Streptococcus pneumoniae
GVLSRTSLRS

SEQ ID NO: 22 - protein, 10 aa, Pseudomonas aeruginosa
WFSVSSNSLY

SEQ ID NO: 23 - protein, 9 aa, Pseudomonas aeruginosa
LSHGLQRSP

SEQ ID NO: 24 - protein, 9 aa, Pseudomonas aeruginosa
GSLNIRLGT

SEQ ID NO: 25 - protein, 12 aa, Streptococcus pneumoniae
FYNLFSVSSATK

SEQ ID NO: 26 - protein, 13 aa, Streptococcus pneumoniae
VRLYVNGVLSRTS

SEQ ID NO: 27 - protein, 15 aa, Streptococcus pneumoniae
KGRVRLYVNGVLSRT

SEQ ID NO: 28 - protein, 15 aa, Pseudomonas aeruginosa
GAQVEVGSLNIRLGT

SEQ ID NO: 29 - protein, 15 aa, Streptococcus pneumoniae
FYNLFSVSSATKKDE

SEQ ID NO: 30 - protein, 15 aa, Pseudomonas aeruginosa
SDWFSVSSNSLYTLS

SEQ ID NO: 31 - protein, 9 aa, Streptococcus pneumoniae
IRNLTVYNR